European Patent Specification EP 4 456 905 B1, published July 30, 2025. Title: Microbial communities. Applicant: MRM Health N.V. The sequence listing filed with the application follows.

SEQUENCE LISTING (9 sequences)

SEQ ID NO: 1 - DNA, 1454 bp, Roseburia inulinivorans
  misc_feature 1..1454: note = Roseburia inulinivorans DSMZ 16841 16S rRNA gene
  source 1..1454: mol_type = other DNA
ttgatcctggctcaggatgaacgctggcggcgtgcttaacacatgcaagtcgaacgaagcacttttacagatttcttcggaatgaagttttagtgactgagtggcggacgggtgagtaacgcgtgggtaacctgcctcacacagggggataacagttggaaacggctgctaataccgcataagcgcacagtaccgcatggtacagtgtgaaaaactccggtggtgtgagatggacccgcgtctgattagctagttggcagggcaacggcctaccaaggcgacgatcagtagccgacctgagagggtgaccggccacattgggactgagacacggcccaaactcctacgggaggcagcagtggggaatattgcacaatgggggaaaccctgatgcagcgacgccgcgtgagcgaagaagtatttcggtatgtaaagctctatcagcagggaagaagaaatgacggtacctgactaagaagcaccggctaaatacgtgccagcagccgcggtaatacgtatggtgcaagcgttatccggatttactgggtgtaaagggagcgcaggcggaaggctaagtctgatgtgaaagcccggggctcaaccccggtactgcattggaaactggtcatctagagtgtcggaggggtaagtggaattcctagtgtagcggtgaaatgcgtagatattaggaggaacaccagtggcgaaggcggcttactggacgataactgacgctgaggctcgaaagcgtggggagcaaacaggattagataccctggtagtccacgccgtaaacgatgaatactaggtgtcggaaagcacagcttttcggtgccgccgcaaacgcattaagtattccacctggggagtacgttcgcaagaatgaaactcaaaggaattgacggggacccgcacaagcggtggagcatgtggtttaattcgaagcaacgcgaagaaccttaccaagtcttgacatccttctgaccggacagtaatgtgtcctttccttcgggacagaagtgacaggtggtgcatggttgtcgtcagctcgtgtcgtgagatgttgggttaagtcccgcaacgagcgcaacccttatccccagtagccagcggttcggacgggcactctgaggagactgccagggataacctggaggaaggtggggatgacgtcaaatcatcatgccccttatgacttgggctacacacgtgctacaatggcgtaaacaaagggaagcgagaccgtgaggtggagcaaatcccaaaaataacgtctcagttcggactgtagtctgcaacccgactacacgaagctggaatcgctagtaatcgcagatcagaatgctgcggtgaatacgttcccgggtcttgtacacaccgcccgtcacaccatgggagttggaaatgcccgaagtcagtgacccaaccgcaaggagggagctgcgaaggcaggt

SEQ ID NO: 2 - DNA, 1433 bp, Akkermansia muciniphila
  misc_feature 1..1433: note = Akkermansia muciniphila DSMZ 22959 16S rRNA gene
  source 1..1433: mol_type = other DNA
aacgaacgctggcggcgtggataagacatgcaagtcgaacgagagaattgctagcttgctaataattctctagtggcgcacgggtgagtaacacgtgagtaacctgcccccgagagcgggatagccctgggaaactgggattaataccgcatagtatcgaaagattaaagcagcaatgcgcttggggatgggctcgcggcctattagttagttggtgaggtaacggctcaccaaggcgatgacgggtagccggtctgagaggatgtccggccacactggaactgagacacggtccagacacctacgggtggcagcagtcgagaatcattcacaatgggggaaaccctgatggtgcgacgccgcgtgggggaatgaaggtcttcggattgtaaacccctgtcatgtgggagcaaattaaaaagatagtaccacaagaggaagagacggctaactctgtgccagcagccgcggtaatacagaggtctcaagcgttgttcggaatcactgggcgtaaagcgtgcgtaggctgtttcgtaagtcgtgtgtgaaaggcgcgggctcaacccgcggacggcacatgatactgcgagactagagtaatggagggggaaccggaattctcggtgtagcagtgaaatgcgtagatatcgagaggaacactcgtggcgaaggcgggttcctggacattaactgacgctgaggcacgaaggccaggggagcgaaagggattagatacccctgtagtcctggcagtaaacggtgcacgcttggtgtgcggggaatcgaccccctgcgtgccggagtaacgcgttaagcgtgccgcctggggagtacggtcgcaagattaaaactcaaagaaattgacggggacccgcacaagcggtggagtatgtggcttaattcgatgcaacgcgaagaaccttacctgggcttgacatgtaatgaacaacatgtgaaagcatgcgactcttcggaggcgttacacaggtgctgcatggccgtcgtcagctcgtgtcgtgagatgtttggttaagtccagcaacgagcgcaacccctgttgccagttaccagcacgtgaaggtggggactctggcgagactgcccagatcaactgggaggaaggtggggacgacgtcaggtcagtatggcccttatgcccagggctgcacacgtactacaatgcccagtacagagggggccgaagccgcgaggcggaggaaatcctaaaaactgggcccagttcggactgtaggctgcaacccgcctacacgaagccggaatcgctagtaatggcgcatcagctacggcgccgtgaatacgttcccgggtcttgtacacaccgcccgtcacatcatggaagctggtcgcacccgaagtatctgaagccaaccgcaaggaggcagggtcctaaggtgagactggtaactgggatg

SEQ ID NO: 3 - DNA, 1456 bp, Anaerostipes caccae
  misc_feature 1..1456: note = Anaerostipes caccae DSMZ 14662 16S rRNA gene
  source 1..1456: mol_type = other DNA
gcgcttaatacatgtcaagtcgaacgaagcatttaggattgaagttttcggatggatttcctatatgactgagtggcggacgggtgagtaacgcgtggggaacctgccctatacagggggataacagctggaaacggctgctaataccgcataagcgcacagaatcgcatgattcagtgtgaaaagccctggcagtataggatggtcccgcgtctgattagctggttggtgaggtaacggctcaccaaggcgacgatcagtagccggcttgagagagtgaacggccacattgggactgagacacggcccaaactcctacgggaggcagcagtggggaatattgcacaatgggggtaaaccctgatgcagcgacgccgcgtgagtgaagaagtatttcggtatgtaaagctctatcagcagggaagaaaacagacggtacctgactaagaagccccggctaactacgtgccagcagccgcggtaatacgtagggggcaagcgttatccggaattactgggtgtaaagggtgcgtaggtggcatggtaagtcagaagtgaaagcccggggcttaaccccgggactgcttttgaaactgtcatgctggagtgcaggagaggtaagcggaattcctagtgtagcggtgaaatgcgtagatattaggaggaacaccagtggcgaaggcggcttactggactgtcactgacactgatgcacgaaagcgtggggagcaaacaggattagataccctggtagtccacgccgtaaacgatgaatactaggtgtcggggccgtagaggcttcggtgccgcagcaaacgcagtaagtattccacctggggagtacgttcgcaagaatgaaactcaaaggaattgacggggacccgcacaagcggtggagcatgtggtttaattcgaagcaacgcgaagaaccttacctggtcttgacatcccaatgaccgaaccttaaccggttttttctttcgagacattggagacaggtggtgcatggttgtcgtcagctcgtgtcgtgagatgttgggttaagtcccgcaacgagcgcaacccctatctttagtagccagcatttaaggtgggcactctagagagactgccagggataacctggaggaaggtggggacgacgtcaaatcatcatgccccttatggccagggctacacacgtgctacaatggcgtaaacaaagggaagcgaagtcgtgaggcgaagcaaatcccagaaataacgtctcagttcggattgtagtctgcaactcgactacatgaagctggaatcgctagtaatcgtgaatcagaatgtcacggtgaatacgttcccgggtcttgtacacaccgcccgtcacaccatgggagtcagtaacgcccgaagtcagtgacccaaccgcaaggagggagctgccgaaggtgggaccgataactggggtgaagtcgtaacaagg

SEQ ID NO: 4 - DNA, 1466 bp, Faecalibacterium prausnitzii
  misc_feature 1..1466: note = Faecalibacterium prausnitzii DSMZ 17677 16S rRNA gene
  source 1..1466: mol_type = other DNA
gttgatcctggctcaggacgaacgctggcggcgcgcctaacacatgcaagtcgaacgagcgagagagagcttgctttctcgagcgagtggcgaacgggtgagtaacgcgtgaggaacctgcctcaaagagggggacaacagttggaaacgactgctaataccgcataagcccacagctcggcatcgagcagagggaaaaggagcaatccgctttgagatggcctcgcgtccgattagctagttggtgaggtaatggcccaccaaggcaacgatcggtagccggactgagaggttgaacggccacattgggactgagacacggcccagactcctacgggaggcagcagtggggaatattgcacaatgggggaaaccctgatgcagcgacgccgcgtggaggaagaaggtcttcggattgtaaactcctgttgttgaggaagataatgacggtactcaacaaggaagtgacggctaactacgtgccagcagccgcggtaaaacgtaggtcacaagcgttgtccggaattactgggtgtaaagggagcgcaggcgggaagacaagttggaagtgaaatctatgggctcaacccataaactgctttcaaaactgtttttcttgagtagtgcagaggtaggcggaattcccggtgtagcggtggaatgcgtagatatcgggaggaacaccagtggcgaaggcggcctactgggcaccaactgacgctgaggctcgaaagtgtgggtagcaaacaggattagataccctggtagtccacaccgtaaacgatgattactaggtgttggaggattgaccccttcagtgccgcagttaacacaataagtaatccacctggggagtacgaccgcaaggttgaaactcaaaggaattgacgggggcccgcacaagcagtggagtatgtggtttaattcgacgcaacgcgaagaaccttaccaagtcttgacatcctgcgacgatgctggaaacagtattttccttcgggacgcagagacaggtggtgcatggttgtcgtcagctcgtgtcgtgagatgttgggttaagtcccgcaacgagcgcaacccttactgtcagttactacgcaagaggactctggcaggactgccgttgacaaaacggaggaaggtggggatgacgtcaaatcatcatgccctttatgacttgggctacacacgtactacaatggcgttaaacaaagagaagcaagaccgcgaggtggagcaaaactcagaaacaacgtcccagttcggactgcaggctgcaactcgcctgcacgaagtcggaattgctagtaatcgtggatcagcatgccacggtgaatacgttcccgggccttgtacacaccgcccgtcacaccatgagagccggggggacccgaagtcggtagtctaaccgcaaggaggacgccgccgaaggtaaaactggtgattggggtgaagtcgtaacaaggtac

SEQ ID NO: 5 - DNA, 1586 bp, Lactiplantibacillus plantarum
  misc_feature 1..1586: note = Lactiplantibacillus plantarum ZJ316 16S rRNA gene
  source 1..1586: mol_type = other DNA
gggacatgctgcagtcgacgattagagtttgatcctggctcaggacgaacgctggcggcgtgcctaatacatgcaagtcgaacgaactctggtattgattggtgcttgcatcatgatttacatttgagtgagtggcgaactggtgagtaacacgtgggaaacctgcccagaagcgggggataacacctggaaacagatgctaataccgcataacaacttggaccgcatggtccgagtttgaaagatggcttcggctatcacttttggatggtcccgcggcgtattagctagatggtgaggtaacggcttaccatggcaatgatacgtagccgacctgagagggtaatcggccacattgggactgagacacggcccaaactcctacgggaggcagcagtagggaatcttccacaatggacgaaagtctgatggagcaacgccgcgtgagtgaagaagggtttcggctcgtaaaactctgttgttaaagaagaacatatctgagagtaactgttcaggtattgacggtatttaaccagaaagccacggctaactacgtgccagcagccgcggtaatacgtaggtggcaagcgttgtccggatttattgggcgtaaagcgagcgcaggcggttttttaagtctgatgtgaaagccttcggctcaaccgaagaagtgcatcggaaactgggaaacttgagtgcagaagaggacagtggaactccatgtgtagcggtgaaatgcgtagatatatggaagaacaccagtggcgaaggcggctgtctggtctgtaactgacgctgaggctcgaaagtatgggtagcaaacaggattagataccctggtagtccataccgtaaacgatgaatgctaagtgttggagggtttccgcccttcagtgctgcagctaacgcattaagcattccgcctggggagtacggccgcaaggctgaaactcaaaggaattgacgggggcccgcacaagcggtggagcatgtggtttaattcgaagctacgcgaagaaccttaccaggtcttgacatactatgcaaatctaagagattagacgttcccttcggggacatggatacaggtggtgcatggttgtcgtcagctcgtgtcgtgagatgttgggttaagtcccgcaacgagcgcaacccttattatcagttgccagcattaagttgggcactctggtgagactgccggtgacaaaccggaggaaggtggggatgacgtcaaatcatcatgccccttatgacctgggctacacacgtgctacaatggatggtacaacgagttgcgaactcgcgagagtaagctaatctcttaaagccattctcagttcggattgtaggctgcaactcgcctacatgaagtcggaatcgctagtaatcgcggatcagcatgccgcggtgaatacgttcccgggccttgtacacaccgcccgtcacaccatgagagtttgtaacacccaaagtcggtggggtaaccttttaggaaccagccgcctaaggtgggacagatgattagggtgaagtcgtaacaaggtaaccaatctctagaggtccccgggaccgagctgacgcaa

SEQ ID NO: 6 - DNA, 1482 bp, Butyricicoccus pullicaecorum
  misc_feature 1..1482: note = Butyricicoccus pullicaecorum LMG 24109 16S rRNA gene
  source 1..1482: mol_type = other DNA
tagtttgatcctggctcaggatgaacgctggcggcgtgcctaacacatgcaagtcgaacggagttgtttgaggaaatccttcgggatggaatcttccaacttagtggcggacgggtgagtaacgcgtgagcaatctgcctttcagagggggataacagccggaaacggctgctaataccgcataatgcattgaattcgcatgtttttgatgccaaagattttatcgctgaaagatgagctcgcgtctgattagctagttggcggggtaacggcccaccaaggcgacgatcagtagccggactgagaggttgaacggccacattgggactgaggacacggcccagactcctaccgggaggcagcagtggggaatattgcgcaatgggggcaaccctgacgcagcaacgccgcgtgattgatgaaggtcttcggattgtaaaaatctttaatcagggacgaaacaaatgacggtacctgaagaataagctccggctaactacgtgccagcagccgcggtaatacgtagggagcaagcgttatccggatttactgggtgtaaagggcgtgtaggcgggcttgtaagttggaagtgaaatctcggggcttaaccccgaaactgctttcaaaactgcgagtcttgagtgatggagaggcaggcggaattcccagtgtagcggtgaaatgcgtagatattgggaggaacaccagtggcgaaggcggcctgctggacattaactgacgctgaggcgcgaaagcgtggggagcaaacaggattagataccctggtagtccacgccgtaaacgatggatactaggtgtgggaggtattgaccccttccgtgccggagttaacacaataagtatcccacctggggagtacggccgcaaggttgaaactcaaaggaattgacgggggcccgcacaagcagtggagtatgtggtttaattcgaagcaacgcgcaagaaccttaccaagtcttgacatcccgatgaccgctcyagagatagggcttttcttcggaacatcggtgacaggtggtgcatggttgtcgtcagctcgtgtcgtgagatgttgggttaagtcccgcaacgagcgcaacccttacgggttagttgctacgcaagagcactctagccggactgccgttgacaaaacggaggaaggtggggacgacgtcaaatcatcatgccccttatgacttgggctacacacgtactacaatggcagtcatacagagggaagcaaaaccgcgaggtggagcaaatccctaaaagctgtcccagttcagattgcaggctgcaactcgcctgcatgaagtcggaattgctagtaatcgcggatcagcatgccgcggtgaatacgttcccgggccttgtacacaccgcccgtcacaccatgagagccggtaatacccgaagtccgtagtctaaccgcaaggaggacgcggccgaaggtaggactggtaattgggacgaagtcgt

SEQ ID NO: 7 - DNA, 1510 bp, Phocaeicola vulgatus
  misc_feature 1..1510: note = Phocaeicola vulgatus LMG17767 16S rRNA gene
  source 1..1510: mol_type = other DNA
tattacaatgaagagtttgatcctggctcaggatgaacgctagctacaggcttaacacatgcaagtcgaggggcagcatggtcttagcttgctaaggccgatggcgaccggcgcacgggtgagtaacacgtatccaacctgccgtctactcttggacagccttctgaaaggaagattaatacaagatggcatcatgagtccgcatgttcacatgattaaaggtattccggtagacgatggggatgcgttccattagatagtaggcggggtaacggcccacctagtcttcgatggataggggttctgagaggaaggtcccccacattggaactgagacacggtccaaactcctacgggaggcagcagtgaggaatattggtcaatgggcgagagcctgaaccagccaagtagcgtgaaggatgactgccctatgggttgtaaacttcttttataaaggaataaagtcgggtatggatacccgtttgcatgtactttatgaataaggatcggctaactccgtgccagcagccgcggtaatacggaggatccgagcgttatccggatttattgggtttaaagggagcgtagatggatgtttaagtcagttgtgaaagtttgcggctcaaccgtaaaattgcagttgatactggatatcttgagtgcagttgaggcaggcggaattcgtggtgtagcggtgaaatgcttagatatcacgaagaactccgattgcgaaggcagcctgctaagctgcaactgacattgaggctcgaaagtgtgggtatcaaacaggattagataccctggtagtccacacggtaaacgatgaatactcgctgtttgcgatatactgcaagcggccaagcgaaagcgttaagtattccacctggggagtacgccggcaacggtgaaactcaaaggaattgacgggggcccgcacaagcggaggaacatgtggtttaattcgatgatacgcgaggaaccttacccgggcttaaattgcagatgaattacggtgaaagccgtaagccgcaaggcatctgtgaaggtgctgcatggttgtcgtcagctcgtgccgtgaggtgtcggcttaagtgccataacgagcgcaacccttgttgtcagttactaacaggttccgctgaggactctgacaagactgccatcgtaagatgtgaggaaggtggggatgacgtcaaatcagcacggcccttacgtccggggctacacacgtgttacaatggggggtacagagggccgctaccacgcgagtggatgccaatccccaaaacctctctcagttcggactggagtctgcaacccgactccacgaagctggattcgctagtaatcgcgcatcagccacggcgcggtgaatacgttcccgggccttgtacacaccgcccgtcaagccatgggagccgggggtacctgaagtgcgtaaccgcgaggagcgccctagggtaaaactggtgactggggctaagtcgtaacaaggtagccgtaccggaag

SEQ ID NO: 8 - DNA, 1500 bp, Veillonella parvula
  misc_feature 1..1500: note = Veillonella parvula DSM 2007 16S rRNA gene
  source 1..1500: mol_type = other DNA
gcgaagctggcggcgtgcttaacacatgcaagtcgaacgaagagcgatggaagcttgcttctatcaatcttagtggcgaacgggtgagtaacgcgtaatcaacctgcccttcagagggggacaacagttggaaacgactgctaataccgcatacgatctaatctcggcatcgaggatagatgaaaggtggcctctacatgtaagctatcactgaaggaggggattgcgtctgattagctagttggaggggtaacggcccaccaaggcgatgatcagtagccggtctgagaggatgaacggccacattgggactgagacacggcccagactcctacgggaggcagcagtggggaatcttccgcaatggacgaaagtctgacggagcaacgccgcgtgagtgatgacggccttcgggttgtaaagctctgttaatcgggacgaaaggccttcttgcgaatagtgagaaggattgacggtaccggaatagaaagccacggctaactacgtgccagcagccgcggtaatacgtaggtggcaagcgttgtccggaattattgggcgtaaagcgcgcgcaggcggatmggtcagtctgtcttaaaagttcggggcttaaccccgtgatgggatggaaactgccaatctagagtatcggagaggaaagtggaattcctagtgtagcggtgaaatgcgtagatattaggaagaacaccagtggcgaaggcgactttctggacgaaaactgacgctgaggcgcgaaagccaggggagcgaacgggattagataccccggtagtcctggccgtaaacgatgggtactaggtgtaggaggtatcgaccccttctgtgccggagttaacgcaataagtaccccgcctggggagtacgaccgcaaggttgaaactcaaaggaattgacgggggcccgcacaagcggtggagtatgtggtttaattcgacgcaacgcgaagaaccttaccaggtcttgacattgatggacagaaccagagatggttcctcttcttcggaagccagaaaacaggtggtgcacggttgtcgtcagctcgtgtcgtgagatgttgggttaagtcccgcaacgagcgcaacccctatcttatgttgccagcactttgggtggggactcatgagagactgccgcagacaatgcggaggaaggcggggatgacgtcaaatcatcatgccccttatgacctgggctacacacgtactacaatgggagttaatagacggaagcgagatcgcgagatggagcaaacccgagaaacactctctcagttcggatcgtaggctgcaactcgcctacgtgaagtcggaatcgctagtaatcgcaggtcagcatactgcggtgaatacgttcccgggccttgtacacaccgcccgtcacaccacgaaagtcggaagtgcccaaagccggtggggtaaccttcgggagccagccgtctaaggtaaagtcgatgattggggtgaagtcgtaacaaggtag

SEQ ID NO: 9 - DNA, 1457 bp, Blautia obeum
  misc_feature 1..1457: note = Blautia obeum DSM 25238 16S rRNA gene
  misc_feature 65..66: note = n is a, c, g, or t
  misc_feature 960: note = n is a, c, g, or t
  source 1..1457: mol_type = other DNA
ggcggcgtgcttaacacatgcaagtcgaacgggaaacctttcattgaagcttcggcagatttggnntgtttctagtggcggacgggtgagtaacgcgtgggtaacctgccttatacagggggataacaaccagaaatggttgctaataccgcataagcgcacaggaccgcatggtctggtgtgaaaaactccggtggtataagatggacccgcgttggattagctagttggcagggtaacggcctaccaaggcgacgatccatagccggcctgagagggtgaacggccacattgggactgagacacggcccagactcctacgggaggcagcagtggggaatattgcacaatgggggaaaccctgatgcagcgacgccgcgtgaaggaagaagtatctcggtatgtaaacttctatcagcagggaagatagtgacggtacctgactaagaagccccggctaactacgtgccagcagccgcggtaatacgtagggggcaagcgttatccggatttactgggtgtaaagggagcgtagacggactggcaagtctgatgtgaaaggcgggggctcaacccctggactgcattggaaactgttagtcttgagtgccggagaggtaagcggaattcctagtgtagcggtgaaatgcgtagatattaggaggaacaccagtggcgaaggcggcttactggacggtaactgacgttgaggctcgaaagcgtggggagcaaacaggattagataccctggtagtccacgccgtaaacgatgattactaggtgttggggagcaaagctcttcggtgccgccgcaaacgcattaagtattccacctggggagtacgttcgcaagaatgaaactcaaaggaattgacggggacccgcacaagcggtggagcatgtggtttaattcgaagcaacgcgaagaaccttaccaagtcttgacatccctctgaccgncccttaaccggatctttccttcgggacaggggagacaggtggtgcatggttgtcgtcagctcgtgtcgtgagatgttgggttaagtcccgcaacgagcgcaacccctatccccagtagccagcagtccggctgggcactctgaggagactgccagggataacctggaggaaggcggggatgacgtcaaatcatcatgccccttatgatttgggctacacacgtgctacaatggcgtaaacaaagggaagcaagcctgcgaaggtaagcaaatcccaaaaataacgtcccagttcggactgcagtctgcaactcgactgcacgaagctggaatcgctagtaatcgcggatcagaatgccgcggtgaatacgttcccgggtcttgtacacaccgcccgtcacaccatgggagtcagtaacgcccgaagtcagtgacctaactgcaaagaaggagctgccgaaggcgggaccgatgactggggtgaagtcgtaacaaggt